European Patent Application EP 4 681 716 A1, published January 21, 2026. Title: COMPOSITION FOR ENHANCING EXERCISE PERFORMANCE, INCREASING MUSCLE MASS, IMPROVING MUSCULAR FUNCTIONS, OR PREVENTING OR TREATING MUSCULAR DISEASE CONTAINING POLYGONUM MULTIFLORUM THUNBERG EXTRACT. Applicant: KOREA INSTITUTE OF SCIENCE AND TECHNOLOGY. The sequence listing filed with the application follows.

SEQUENCE LISTING (14 sequences)

SEQ ID NO: 1 - DNA, 20 bp, synthetic construct
  misc_feature 1..20: note = Myod_primer F
  source 1..20: mol_type = other DNA
catagacttgacaggccccg

SEQ ID NO: 2 - DNA, 20 bp, synthetic construct
  misc_feature 1..20: note = Myod_primer R
  source 1..20: mol_type = other DNA
cgggtccaggtcctcaaaaa

SEQ ID NO: 3 - DNA, 20 bp, synthetic construct
  misc_feature 1..20: note = Myog_primer F
  source 1..20: mol_type = other DNA
agctatccggttccaaagcc

SEQ ID NO: 4 - DNA, 20 bp, synthetic construct
  misc_feature 1..20: note = Myog_primer R
  source 1..20: mol_type = other DNA
gcacaggagaccttggtcag

SEQ ID NO: 5 - DNA, 20 bp, synthetic construct
  misc_feature 1..20: note = Myh2_primer F
  source 1..20: mol_type = other DNA
agcgaagagtaaggctgtcc

SEQ ID NO: 6 - DNA, 19 bp, synthetic construct
  misc_feature 1..19: note = Myh2_primer R
  source 1..19: mol_type = other DNA
aggcgcatgaccaaaggtt

SEQ ID NO: 7 - DNA, 20 bp, synthetic construct
  misc_feature 1..20: note = Myf5_primer F
  source 1..20: mol_type = other DNA
tccaggtattcccacctgct

SEQ ID NO: 8 - DNA, 20 bp, synthetic construct
  misc_feature 1..20: note = Myf5_primer R
  source 1..20: mol_type = other DNA
tcagctttgtgtgctccgaa

SEQ ID NO: 9 - DNA, 20 bp, synthetic construct
  misc_feature 1..20: note = Myf6_primer F
  source 1..20: mol_type = other DNA
acagatcgtcggaaagcagc

SEQ ID NO: 10 - DNA, 20 bp, synthetic construct
  misc_feature 1..20: note = Myf6_primer R
  source 1..20: mol_type = other DNA
cactccgcagaatctccacc

SEQ ID NO: 11 - DNA, 20 bp, synthetic construct
  misc_feature 1..20: note = Nfr1_primer F
  source 1..20: mol_type = other DNA
cccgtgttcctttgtggtga

SEQ ID NO: 12 - DNA, 20 bp, synthetic construct
  misc_feature 1..20: note = Nfr1_primer R
  source 1..20: mol_type = other DNA
attccatgctctgctgctgg

SEQ ID NO: 13 - DNA, 20 bp, synthetic construct
  misc_feature 1..20: note = Ucp3_primer F
  source 1..20: mol_type = other DNA
gttttgcggacctcctcact

SEQ ID NO: 14 - DNA, 20 bp, synthetic construct
  misc_feature 1..20: note = Ucp3_primer R
  source 1..20: mol_type = other DNA
ctctgtgcgcaccatagtca